European Patent Application EP 4 501 960 A1, published February 5, 2025. Title: MONOCLONAL ANTIBODY AGAINST HLA-G MOLECULES AND USE THEREOF. Applicant: TAIZHOU ENZE MEDICAL CENTER (GROUP). Application EP 22934556.6. The sequence listing filed with the application follows.

SEQUENCE LISTING (19 sequences)

SEQ ID NO: 1 - protein, 112 aa, Artificial Sequence
  Synthetic: HybridomaYWHG-1)
DIVITQDELSLTVSLGDQASISCRTSQSFVHSNGNIYLEWFLQKPGQSPKLLIYKVSSRFSGVPDRFSGSGSGTDFTLKISRVEAEDLGIYYCFQGSHVPPTFGGGTKLEIK

SEQ ID NO: 2 - protein, 11 aa, Artificial Sequence
  Synthetic: HybridomaYWHG-1)
QSFVHSNGNIY

SEQ ID NO: 3 - protein, 3 aa, Artificial Sequence
  Synthetic: HybridomaYWHG-1)
KVS

SEQ ID NO: 4 - protein, 9 aa, Artificial Sequence
  Synthetic: HybridomaYWHG-1)
FQGSHVPPT

SEQ ID NO: 5 - protein, 114 aa, Artificial Sequence
  Synthetic: HybridomaYWHG-1)
QLQESGTVLVRPGASVKLSCKASGYIFTSYWINWVKQRPGQGLEWIGNIYPSDSYTNFNQKFEDKATLTVDTSSSTAYMQFSSPTSEDSAVYYCTRFGYPFDYWGQGTTLTVSS

SEQ ID NO: 6 - protein, 8 aa, Artificial Sequence
  Synthetic: HybridomaYWHG-1)
GYIFTSYW

SEQ ID NO: 7 - protein, 8 aa, Artificial Sequence
  Synthetic: HybridomaYWHG-1)
IYPSDSYT

SEQ ID NO: 8 - protein, 9 aa, Artificial Sequence
  Synthetic: HybridomaYWHG-1)
TRFGYPFDY

SEQ ID NO: 9 - protein, 26 aa, Artificial Sequence
  Synthetic: HybridomaYWHG-1)
DIVITQDELSLTVSLGDQASISCRTS

SEQ ID NO: 10 - protein, 17 aa, Artificial Sequence
  Synthetic: HybridomaYWHG-1)
LEWFLQKPGQSPKLLIY

SEQ ID NO: 11 - protein, 36 aa, Artificial Sequence
  Synthetic: HybridomaYWHG-1)
SRFSGVPDRFSGSGSGTDFTLKISRVEAEDLGIYYC

SEQ ID NO: 12 - protein, 10 aa, Artificial Sequence
  Synthetic: HybridomaYWHG-1)
FGGGTKLEIK

SEQ ID NO: 13 - protein, 23 aa, Artificial Sequence
  Synthetic: HybridomaYWHG-1)
QLQESGTVLVRPGASVKLSCKAS

SEQ ID NO: 14 - protein, 17 aa, Artificial Sequence
  Synthetic: HybridomaYWHG-1)
INWVKQRPGQGLEWIGN

SEQ ID NO: 15 - protein, 38 aa, Artificial Sequence
  Synthetic: HybridomaYWHG-1)
NFNQKFEDKATLTVDTSSSTAYMQFSSPTSEDSAVYYC

SEQ ID NO: 16 - protein, 11 aa, Artificial Sequence
  Synthetic: HybridomaYWHG-1)
WGQGTTLTVSS

SEQ ID NO: 17 - DNA, 334 bp, Artificial Sequence
  Synthetic: HybridomaYWHG-1)
gatatcgtgataacccaagatgaactctccctgactgtcagtcttggagatcaggcctccatctcttgcagaactagtcagagttttgtacatagtaatggaaacatctatttagaatggttcctgcgaaaccaggccagtctccaaaactcctgatctacaaagtttccagccgattttctggggtcccagacaggttcagtggcagtggatcagggacagatttcacactcaagatcagcagagtggaggctaggatctgggaatttattactgctttcaaggttcacatgttcctccgacgttcggtggaggcaccaagctggaaatcaaa

SEQ ID NO: 18 - DNA, 340 bp, Artificial Sequence
  Synthetic: HybridomaYWHG-1)
cagctgcaggagtctgggactgttctggtgaggcctggggcttcagtgaagctgtcctgcaaggcttctggctacattttcaccagctactggataaactgggtgaagcagaggcctggacaaggcctgagtggatcggaaatatttatccttctgatagttatactaacttcaatcaaaagttcgaggacaaggccacattgactgtagacacatcctccagcacagcctacatgcagttcagcagcccgacactgaggactctgcggtctattattgtacaagatttggttacccctttgactactggggccaaggcacaactctcacagtctcctca

SEQ ID NO: 19 - protein, 20 aa, Artificial Sequence
  Synthetic: HybridomaYWHG-1)
QTDRMNLQTLRGYYNQSEAS